European Patent Application EP 4 144 372 A2, published March 8, 2023. Title: ANTIBODIES AGAINST SIGNAL-REGULATORY PROTEIN ALPHA AND METHODS OF USE. Applicant: ALX Oncology Inc. Application EP TBC, filed March 20, 2019. The sequence listing filed with the application follows.

SEQUENCE LISTING (140 sequences)

SEQ ID NO: 1 - protein, 348 aa, synthetic construct
  SOURCE 1..348
  REGION 1..348: NOTE = Synthetic Construct
EEELQVIQPDKSVLVAAGETATLRCTATSLIPVGPIQWFRGAGPGRELIYNQKEGHFPRVTTVSDLTKRNNMDFSIRIGNITPADAGTYYCVKFRKGSPDDVEFKSGAGTELSVRAKPSESKYGPPCPPCPAPEFLGGPSVFLFPPKPKDTLMISRTPEVTCVVVDVSQEDPEVQFNWYVDGVEVHNAKTKPREEQFNSTYRVVSVLTVLHQDWLNGKEYKCKVSNKGLPSSIEKTISKAKGQPREPQVYTLPPSQEEMTKNQVSLTCLVKGFYPSDIAVEWESNGQPENNYKTTPPVLDSDGSFFLYSRLTVDKSRWQEGNVFSCSVMHEALHNHYTQKSLSLSLGK

SEQ ID NO: 2 - protein, 347 aa, synthetic construct
  SOURCE 1..347
  REGION 1..347: NOTE = Synthetic Construct
EEELQVIQPDKSVSVAAGESAILHCTVTSLIPVGPIQWFRGAGPARELIYNQKEGHFPRVTTVSESTKRENMDFSISISNITPADAGTYYCVKFRKGSPDTEFKSGAGTELSVRAKPSESKYGPPCPPCPAPEFLGGPSVFLFPPKPKDTLMISRTPEVTCVVVDVSQEDPEVQFNWYVDGVEVHNAKTKPREEQFNSTYRVVSVLTVLHQDWLNGKEYKCKVSNKGLPSSIEKTISKAKGQPREPQVYTLPPSQEEMTKNQVSLTCLVKGFYPSDIAVEWESNGQPENNYKTTPPVLDSDGSFFLYSRLTVDKSRWQEGNVFSCSVMHEALHNHYTQKSLSLSLGK

SEQ ID NO: 3 - protein, 346 aa, synthetic construct
  SOURCE 1..346
  REGION 1..346: NOTE = Synthetic Construct
KELKVTQPEKSVSVAAGDSTVLNCTLTSLLPVGPIKWYRGVGQSRLLIYSFTGEHFPRVTNVSDATKRNNMDFSIRISNVTPEDAGTYYCVKFQKGPSEPDTEIQSGGGTEVYVLAKPSDKTHTCPPCPAPEAAGAPSVFLFPPKPKDTLMISRTPEVTCVVVDVSHEDPEVKFNWYVDGVEVHNAKTKPREEQYASTYRVVSVLTVLHQDWLNGKEYKCKVSNKALPAPIEKTISKAKGQPREPQVYTLPPSREEMTKNQVSLTCLVKGFYPSDIAVEWESNGQPENNYKTTPPVLDSDGSFFLYSKLTVDKSRWQQGNVFSCSVMHEALHNHYTQKSLSLSPGK

SEQ ID NO: 4 - protein, 342 aa, synthetic construct
  SOURCE 1..342
  REGION 1..342: NOTE = Synthetic Construct
TEVKVIQPEKSVSVAAGDSTVLNCTLTSLLPVGPIRWYRGVGQSRQLIYSFTTEHFPRVTNVSDATKRSNLDFSIRISNVTPEDAGTYYCVKFQRGSPDTEIQSGGGTEVYVLAKDKTHTCPPCPAPEAAGAPSVFLFPPKPKDTLMISRTPEVTCVVVDVSHEDPEVKFNWYVDGVEVHNAKTKPREEQYASTYRVVSVLTVLHQDWLNGKEYKCKVSNKALPAPIEKTISKAKGQPREPQVYTLPPSREEMTKNQVSLTCLVKGFYPSDIAVEWESNGQPENNYKTTPPVLDSDGSFFLYSKLTVDKSRWQQGNVFSCSVMHEALHNHYTQKSLSLSPGK

SEQ ID NO: 5 - protein, 119 aa, Homo sapiens
  SOURCE 1..119
EEELQVIQPDKSVLVAAGETATLRCTATSLIPVGPIQWFRGAGPGRELIYNQKEGHFPRVTTVSDLTKRNNMDFSIRIGNITPADAGTYYCVKFRKGSPDDVEFKSGAGTELSVRAKPS

SEQ ID NO: 6 - protein, 118 aa, Homo sapiens
  SOURCE 1..118
EEELQVIQPDKSVSVAAGESAILHCTVTSLIPVGPIQWFRGAGPARELIYNQKEGHFPRVTTVSESTKRENMDFSISISNITPADAGTYYCVKFRKGSPDTEFKSGAGTELSVRAKPS

SEQ ID NO: 7 - protein, 119 aa, Mus musculus
  SOURCE 1..119
KELKVTQPEKSVSVAAGDSTVLNCTLTSLLPVGPIKWYRGVGQSRLLIYSFTGEHFPRVTNVSDATKRNNMDFSIRISNVTPEDAGTYYCVKFQKGPSEPDTEIQSGGGTEVYVLAKPS

SEQ ID NO: 8 - protein, 115 aa, Mus musculus
  SOURCE 1..115
TEVKVIQPEKSVSVAAGDSTVLNCTLTSLLPVGPIRWYRGVGQSRQLIYSFTTEHFPRVTNVSDATKRSNLDFSIRISNVTPEDAGTYYCVKFQRGSPDTEIQSGGGTEVYVLAK

SEQ ID NO: 9 - protein, 117 aa, Mus musculus
  SOURCE 1..117
KELKVTQPEKSVSVAAGDSTVLNCTLTSLLPVGPIRWYRGVGPSRLLIYSFAGEYVPRIRNVSDTTKRNNMDFSIRISNVTPADAGIYYCVKFQKGSSEPDTEIQSGGGTEVYVLAK

SEQ ID NO: 10 - protein, 117 aa, Mus musculus
  SOURCE 1..117
TEVKVTQPEKSVSVAAGDSTILNCTVTSLLPVGPIRWYRGVGQSRLLIYSFTGEHFPRIRNVSDTTKRNNMDFSIRISNVTPEDAGTYYCVKFQRGSSEPDTEIQSGGGTEVYVLAK

SEQ ID NO: 11 - protein, 118 aa, Macaca fascicularis
  SOURCE 1..118
EEELQVIQPEKSVSVAAGESATLNCTATSLIPVGPIQWFRGVGPGRELIYHQKEGHFPRVTPVSDPTKRNNMDFSIRISNITPADAGTYYCVKFRKGSPDVELKSGAGTELSVRAKPS

SEQ ID NO: 12 - protein, 118 aa, Macaca fascicularis
  SOURCE 1..118
EEELQVIQPEKSVSVAAGDSATLNCTVSSLIPVGPIQWFRGAGPGRELIYNLKEGHFPRVTAVSDPTKRNNMDFSIRISNITPADAGTYYCVKFRKGSPDVELKSGAGTELSVRAKPS

SEQ ID NO: 13 - protein, 119 aa, Homo sapiens
  SOURCE 1..119
EDELQVIQPEKSVSVAAGESATLRCAMTSLIPVGPIMWFRGAGAGRELIYNQKEGHFPRVTTVSELTKRNNLDFSISISNITPADAGTYYCVKFRKGSPDDVEFKSGAGTELSVRAKPS

SEQ ID NO: 14 - protein, 119 aa, Homo sapiens
  SOURCE 1..119
EEELQVIQPDKSISVAAGESATLHCTVTSLIPVGPIQWFRGAGPGRELIYNQKEGHFPRVTTVSDLTKRNNMDFSIRISNITPADAGTYYCVKFRKGSPDHVEFKSGAGTELSVRAKPS

SEQ ID NO: 15 - protein, 119 aa, Homo sapiens
  SOURCE 1..119
EEELQMIQPEKLLLVTVGKTATLHCTVTSLLPVGPVLWFRGVGPGRELIYNQKEGHFPRVTTVSDLTKRNNMDFSIRISSITPADVGTYYCVKFRKGSPENVEFKSGPGTEMALGAKPS

SEQ ID NO: 16 - protein, 117 aa, synthetic construct
  SOURCE 1..117
  REGION 1..117: NOTE = Synthetic Construct
QLLFNKTKSVEFTFSNDTVVIPCFVTNMEAQNTTEVYVKWKFKGRDIYTFDGALNKSTVPTDFSSAKIEVSQLLKGDASLKMDKSDAVSHTGNYTCEVTELTREGETIIELKYRVVS

SEQ ID NO: 17 - protein, 118 aa, synthetic construct
  SOURCE 1..118
  REGION 1..118: NOTE = Synthetic Construct
DVQLVESGGGVVRPGESLRLSCAASGFTFSSNAMSWVRQAPGKGLEWLAGISAGGSDTYYPASVKGRFTISRDNSKNTLYLQMNTLTAEDTAVYYCARETWNHLFDYWGLGTLVTVSS

SEQ ID NO: 18 - protein, 107 aa, synthetic construct
  SOURCE 1..107
  REGION 1..107: NOTE = Synthetic Construct
ALTQPASVSANPGETVEITCSGGSYSSYYYAWYQQKSPGSAPVTLIYSDDKRPSNIPSRFSGSASGSTATLTITGVRAEDEAVYFCGGYDQSSYTNPFGAGTTLTVL

SEQ ID NO: 19 - protein, 5 aa, synthetic construct
  SOURCE 1..5
  REGION 1..5: NOTE = Synthetic Construct
SNAMS

SEQ ID NO: 20 - protein, 17 aa, synthetic construct
  SOURCE 1..17
  REGION 1..17: NOTE = Synthetic Construct
GISAGGSDTYYPASVKG

SEQ ID NO: 21 - protein, 9 aa, synthetic construct
  SOURCE 1..9
  REGION 1..9: NOTE = Synthetic Construct
ETWNHLFDY

SEQ ID NO: 22 - protein, 11 aa, synthetic construct
  SOURCE 1..11
  REGION 1..11: NOTE = Synthetic Construct
SGGSYSSYYYA

SEQ ID NO: 23 - protein, 7 aa, synthetic construct
  SOURCE 1..7
  REGION 1..7: NOTE = Synthetic Construct
SDDKRPS

SEQ ID NO: 24 - protein, 11 aa, synthetic construct
  SOURCE 1..11
  REGION 1..11: NOTE = Synthetic Construct
GGYDQSSYTNP

SEQ ID NO: 25 - protein, 108 aa, synthetic construct
  SOURCE 1..108
  REGION 1..108: NOTE = Synthetic Construct
SYELTQPPSVSVSPGQTARITCSGGSYSSYYYAWYQQKPGQAPVTLIYSDDKRPSNIPERFSGSSSGTTVTLTISGVQAEDEADYYCGGYDQSSYTNPFGGGTKLTVL

SEQ ID NO: 26 - protein, 118 aa, synthetic construct
  SOURCE 1..118
  REGION 1..118: NOTE = Synthetic Construct
EVQLVESGGGVVQPGGSLRLSCAASGFTFSSNAMSWVRQAPGKGLEWVAGISAGGSDTYYPASVKGRFTISRDNSKNTLYLQMNSLRAEDTAVYYCARETWNHLFDYWGQGTLVTVSS

SEQ ID NO: 27 - protein, 22 aa, synthetic construct
  SOURCE 1..22
  REGION 1..22: NOTE = Synthetic Construct
SYELTQPPSVSVSPGQTARITC

SEQ ID NO: 28 - protein, 15 aa, synthetic construct
  SOURCE 1..15
  REGION 1..15: NOTE = Synthetic Construct
WYQQKPGQAPVTLIY

SEQ ID NO: 29 - protein, 32 aa, synthetic construct
  SOURCE 1..32
  REGION 1..32: NOTE = Synthetic Construct
NIPERFSGSSSGTTVTLTISGVQAEDEADYYC

SEQ ID NO: 30 - protein, 10 aa, synthetic construct
  SOURCE 1..10
  REGION 1..10: NOTE = Synthetic Construct
FGGGTKLTVL

SEQ ID NO: 31 - protein, 329 aa, synthetic construct
  SOURCE 1..329
  REGION 1..329: NOTE = Synthetic Construct
ASTKGPSVFPLAPSSKSTSGGTAALGCLVKDYFPEPVTVSWNSGALTSGVHTFPAVLQSSGLYSLSSVVTVPSSSLGTQTYICNVNHKPSNTKVDKKVEPKSCDKTHTCPPCPAPELLGGPSVFLFPPKPKDTLMISRTPEVTCVVVDVSHEDPEVKFNWYVDGVEVHNAKTKPREEQYNSTYRVVSVLTVLHQDWLNGKEYKCKVSNKALPAPIEKTISKAKGQPREPQVYTLPPSREEMTKNQVSLTCLVKGFYPSDIAVEWESNGQPENNYKTTPPVLDSDGSFFLYSKLTVDKSRWQQGNVFSCSVMHEALHNHYTQKSLSLSPG

SEQ ID NO: 32 - protein, 329 aa, synthetic construct
  SOURCE 1..329
  REGION 1..329: NOTE = Synthetic Construct
ASTKGPSVFPLAPSSKSTSGGTAALGCLVKDYFPEPVTVSWNSGALTSGVHTFPAVLQSSGLYSLSSVVTVPSSSLGTQTYICNVNHKPSNTKVDKKVEPKSCDKTHTCPPCPAPEAAGAPSVFLFPPKPKDTLMISRTPEVTCVVVDVSHEDPEVKFNWYVDGVEVHNAKTKPREEQYASTYRVVSVLTVLHQDWLNGKEYKCKVSNKALPAPIEKTISKAKGQPREPQVYTLPPSREEMTKNQVSLTCLVKGFYPSDIAVEWESNGQPENNYKTTPPVLDSDGSFFLYSKLTVDKSRWQQGNVFSCSVMHEALHNHYTQKSLSLSPG

SEQ ID NO: 33 - protein, 325 aa, synthetic construct
  SOURCE 1..325
  REGION 1..325: NOTE = Synthetic Construct
ASTKGPSVFPLAPCSRSTSESTAALGCLVKDYFPEPVTVSWNSGALTSGVHTFPAVLQSSGLYSLSSVVTVPSSNFGTQTYTCNVDHKPSNTKVDKTVERKCCVECPPCPAPPVAGPSVFLFPPKPKDTLMISRTPEVTCVVVDVSHEDPEVQFNWYVDGVEVHNAKTKPREEQFNSTFRVVSVLTVVHQDWLNGKEYKCKVSNKGLPAPIEKTISKTKGQPREPQVYTLPPSREEMTKNQVSLTCLVKGFYPSDIAVEWESNGQPENNYKTTPPMLDSDGSFFLYSKLTVDKSRWQQGNVFSCSVMHEALHNHYTQKSLSLSPG

SEQ ID NO: 34 - protein, 325 aa, synthetic construct
  SOURCE 1..325
  REGION 1..325: NOTE = Synthetic Construct
ASTKGPSVFPLAPCSRSTSESTAALGCLVKDYFPEPVTVSWNSGALTSGVHTFPAVLQSSGLYSLSSVVTVPSSNFGTQTYTCNVDHKPSNTKVDKTVERKCCVECPPCPAPPVAGPSVFLFPPKPKDTLMISRTPEVTCVVVDVSHEDPEVQFNWYVDGVEVHNAKTKPREEQFNSTFRVVSVLTVVHQDWLNGKEYKCKVSNKGLPSSIEKTISKTKGQPREPQVYTLPPSREEMTKNQVSLTCLVKGFYPSDIAVEWESNGQPENNYKTTPPMLDSDGSFFLYSKLTVDKSRWQQGNVFSCSVMHEALHNHYTQKSLSLSPG

SEQ ID NO: 35 - protein, 326 aa, synthetic construct
  SOURCE 1..326
  REGION 1..326: NOTE = Synthetic Construct
ASTKGPSVFPLAPCSRSTSESTAALGCLVKDYFPEPVTVSWNSGALTSGVHTFPAVLQSSGLYSLSSVVTVPSSSLGTKTYTCNVDHKPSNTKVDKRVESKYGPPCPPCPAPEFLGGPSVFLFPPKPKDTLMISRTPEVTCVVVDVSQEDPEVQFNWYVDGVEVHNAKTKPREEQFNSTYRVVSVLTVLHQDWLNGKEYKCKVSNKGLPSSIEKTISKAKGQPREPQVYTLPPSQEEMTKNQVSLTCLVKGFYPSDIAVEWESNGQPENNYKTTPPVLDSDGSFFLYSRLTVDKSRWQEGNVFSCSVMHEALHNHYTQKSLSLSLG

SEQ ID NO: 36 - protein, 107 aa, synthetic construct [sequence omitted]

SEQ ID NO: 37 - protein, 106 aa, synthetic construct
  SOURCE 1..106
  REGION 1..106: NOTE = Synthetic Construct
GQPKANPTVTLFPPSSEELQANKATLVCLISDFYPGAVTVAWKADGSPVKAGVETTKPSKQSNNKYAASSYLSLTPEQWKSHRSYSCQVTHEGSTVEKTVAPTECS

SEQ ID NO: 38 - protein, 106 aa, synthetic construct
  SOURCE 1..106
  REGION 1..106: NOTE = Synthetic Construct
GQPKAAPSVTLFPPSSEELQANKATLVCLISDFYPGAVTVAWKADSSPVKAGVETTTPSKQSNNKYAASSYLSLTPEQWKSHRSYSCQVTHEGSTVEKTVAPTECS

SEQ ID NO: 39 - protein, 108 aa, synthetic construct
  SOURCE 1..108
  REGION 1..108: NOTE = Synthetic Construct
SYELTQPPSVSVSPGQTARITCSGGSYSSYYYAWYQQKPGQAPVTLIYSDDKRPSNIPERFSGSSSGTTVTLTISGVQAEDEADYYCGGYDQSSYTNPFGTGTKVTVL

SEQ ID NO: 40 - protein, 108 aa, synthetic construct
  SOURCE 1..108
  REGION 1..108: NOTE = Synthetic Construct
SYELTQPPSVSVSPGQTARITCSGGSYSSYYYAWYQQKPGQAPVTLIYSDDKRPSNIPERFSGSSSGTTVTLTISGVQAEDEADYYCGGYDQSSYTNPFGGGTQLTVL

SEQ ID NO: 41 - protein, 108 aa, synthetic construct
  SOURCE 1..108
  REGION 1..108: NOTE = Synthetic Construct
SYELTQPPSVSVSPGQTARITCSGGSYSSYYYAWYQQKPGQAPVTLIYSDDKRPSNIPERFSGSSSGTTVTLTISGVQAEDEADYYCGGYDQSSYTNPFGGGTRLTVL

SEQ ID NO: 42 - protein, 106 aa, synthetic construct; identical to SEQ ID NO: 37
  SOURCE 1..106
  REGION 1..106: NOTE = Synthetic Construct

SEQ ID NO: 43 - protein, 106 aa, synthetic construct
  SOURCE 1..106
  REGION 1..106: NOTE = Synthetic Construct
GQPKANPTVTLFPPSSEELQANKATLVCLISDFYPGAVTVAWKADGSPVKAGVETTKPSKQSNDKYAASSYLSLTPEQWKSHRSYSCQVTHEGSTVEKTVAPTECS

SEQ ID NO: 44 - protein, 106 aa, synthetic construct
  SOURCE 1..106
  REGION 1..106: NOTE = Synthetic Construct
GQPKANPTVTLFPPSSEELQANKATLVCLISDFYPGAVTVAWKADGSPVKAGVETTKPSKQSDNKYAASSYLSLTPEQWKSHRSYSCQVTHEGSTVEKTVAPTECS

SEQ ID NO: 45 - protein, 106 aa, synthetic construct
  SOURCE 1..106
  REGION 1..106: NOTE = Synthetic Construct
GQPKANPTVTLFPPSSEELQANKATLVCLISDFYPGAVTVAWKADGSPVKAGVETTKPSKQSDSKYAASSYLSLTPEQWKSHRSYSCQVTHEGSTVEKTVAPTECS

SEQ ID NO: 46 - protein, 106 aa, synthetic construct
  SOURCE 1..106
  REGION 1..106: NOTE = Synthetic Construct
GQPKANPTVTLFPPSSEELQANKATLVCLISDFYPGAVTVAWKADGSPVKAGVETTKPSKQSSDKYAASSYLSLTPEQWKSHRSYSCQVTHEGSTVEKTVAPTECS

SEQ ID NO: 47 - protein, 214 aa, synthetic construct
  SOURCE 1..214
  REGION 1..214: NOTE = Synthetic Construct
SYELTQPPSVSVSPGQTARITCSGGSYSSYYYAWYQQKPGQAPVTLIYSDDKRPSNIPERFSGSSSGTTVTLTISGVQAEDEADYYCGGYDQSSYTNPFGGGTKLTVLGQPKANPTVTLFPPSSEELQANKATLVCLISDFYPGAVTVAWKADGSPVKAGVETTKPSKQSNNKYAASSYLSLTPEQWKSHRSYSCQVTHEGSTVEKTVAPTECS

SEQ ID NO: 48 - protein, 214 aa, synthetic construct
  SOURCE 1..214
  REGION 1..214: NOTE = Synthetic Construct
SYELTQPPSVSVSPGQTARITCSGGSYSSYYYAWYQQKPGQAPVTLIYSDDKRPSNIPERFSGSSSGTTVTLTISGVQAEDEADYYCGGYDQSSYTNPFGGGTKLTVLGQPKANPTVTLFPPSSEELQANKATLVCLISDFYPGAVTVAWKADGSPVKAGVETTKPSKQSNDKYAASSYLSLTPEQWKSHRSYSCQVTHEGSTVEKTVAPTECS

SEQ ID NO: 49 - protein, 214 aa, synthetic construct
  SOURCE 1..214
  REGION 1..214: NOTE = Synthetic Construct
SYELTQPPSVSVSPGQTARITCSGGSYSSYYYAWYQQKPGQAPVTLIYSDDKRPSNIPERFSGSSSGTTVTLTISGVQAEDEADYYCGGYDQSSYTNPFGGGTKLTVLGQPKANPTVTLFPPSSEELQANKATLVCLISDFYPGAVTVAWKADGSPVKAGVETTKPSKQSDNKYAASSYLSLTPEQWKSHRSYSCQVTHEGSTVEKTVAPTECS

SEQ ID NO: 50 - protein, 214 aa, synthetic construct
  SOURCE 1..214
  REGION 1..214: NOTE = Synthetic Construct
SYELTQPPSVSVSPGQTARITCSGGSYSSYYYAWYQQKPGQAPVTLIYSDDKRPSNIPERFSGSSSGTTVTLTISGVQAEDEADYYCGGYDQSSYTNPFGGGTKLTVLGQPKANPTVTLFPPSSEELQANKATLVCLISDFYPGAVTVAWKADGSPVKAGVETTKPSKQSDSKYAASSYLSLTPEQWKSHRSYSCQVTHEGSTVEKTVAPTECS

SEQ ID NO: 51 - protein, 214 aa, synthetic construct
  SOURCE 1..214
  REGION 1..214: NOTE = Synthetic Construct
SYELTQPPSVSVSPGQTARITCSGGSYSSYYYAWYQQKPGQAPVTLIYSDDKRPSNIPERFSGSSSGTTVTLTISGVQAEDEADYYCGGYDQSSYTNPFGGGTKLTVLGQPKANPTVTLFPPSSEELQANKATLVCLISDFYPGAVTVAWKADGSPVKAGVETTKPSKQSSDKYAASSYLSLTPEQWKSHRSYSCQVTHEGSTVEKTVAPTECS

SEQ ID NO: 52 - protein, 214 aa, synthetic construct
  SOURCE 1..214
  REGION 1..214: NOTE = Synthetic Construct
SYELTQPPSVSVSPGQTARITCSGGSYSSYYYAWYQQKPGQAPVTLIYSDDKRPSNIPERFSGSSSGTTVTLTISGVQAEDEADYYCGGYDQSSYTNPFGTGTKVTVLGQPKANPTVTLFPPSSEELQANKATLVCLISDFYPGAVTVAWKADGSPVKAGVETTKPSKQSDSKYAASSYLSLTPEQWKSHRSYSCQVTHEGSTVEKTVAPTECS

SEQ ID NO: 53 - protein, 214 aa, synthetic construct
  SOURCE 1..214
  REGION 1..214: NOTE = Synthetic Construct
SYELTQPPSVSVSPGQTARITCSGGSYSSYYYAWYQQKPGQAPVTLIYSDDKRPSNIPERFSGSSSGTTVTLTISGVQAEDEADYYCGGYDQSSYTNPFGTGTKVTVLGQPKANPTVTLFPPSSEELQANKATLVCLISDFYPGAVTVAWKADGSPVKAGVETTKPSKQSSDKYAASSYLSLTPEQWKSHRSYSCQVTHEGSTVEKTVAPTECS

SEQ ID NO: 54 - protein, 214 aa, synthetic construct
  SOURCE 1..214
  REGION 1..214: NOTE = Synthetic Construct
SYELTQPPSVSVSPGQTARITCSGGSYSSYYYAWYQQKPGQAPVTLIYSDDKRPSNIPERFSGSSSGTTVTLTISGVQAEDEADYYCGGYDQSSYTNPFGGGTQLTVLGQPKANPTVTLFPPSSEELQANKATLVCLISDFYPGAVTVAWKADGSPVKAGVETTKPSKQSDSKYAASSYLSLTPEQWKSHRSYSCQVTHEGSTVEKTVAPTECS

SEQ ID NO: 55 - protein, 214 aa, synthetic construct
  SOURCE 1..214
  REGION 1..214: NOTE = Synthetic Construct
SYELTQPPSVSVSPGQTARITCSGGSYSSYYYAWYQQKPGQAPVTLIYSDDKRPSNIPERFSGSSSGTTVTLTISGVQAEDEADYYCGGYDQSSYTNPFGGGTQLTVLGQPKANPTVTLFPPSSEELQANKATLVCLISDFYPGAVTVAWKADGSPVKAGVETTKPSKQSSDKYAASSYLSLTPEQWKSHRSYSCQVTHEGSTVEKTVAPTECS

SEQ ID NO: 56 - protein, 214 aa, synthetic construct
  SOURCE 1..214
  REGION 1..214: NOTE = Synthetic Construct
SYELTQPPSVSVSPGQTARITCSGGSYSSYYYAWYQQKPGQAPVTLIYSDDKRPSNIPERFSGSSSGTTVTLTISGVQAEDEADYYCGGYDQSSYTNPFGGGTRLTVLGQPKANPTVTLFPPSSEELQANKATLVCLISDFYPGAVTVAWKADGSPVKAGVETTKPSKQSDSKYAASSYLSLTPEQWKSHRSYSCQVTHEGSTVEKTVAPTECS

SEQ ID NO: 57 - protein, 214 aa, synthetic construct
  SOURCE 1..214
  REGION 1..214: NOTE = Synthetic Construct
SYELTQPPSVSVSPGQTARITCSGGSYSSYYYAWYQQKPGQAPVTLIYSDDKRPSNIPERFSGSSSGTTVTLTISGVQAEDEADYYCGGYDQSSYTNPFGGGTRLTVLGQPKANPTVTLFPPSSEELQANKATLVCLISDFYPGAVTVAWKADGSPVKAGVETTKPSKQSSDKYAASSYLSLTPEQWKSHRSYSCQVTHEGSTVEKTVAPTECS

SEQ ID NO: 58 - protein, 447 aa, synthetic construct
  SOURCE 1..447
  REGION 1..447: NOTE = Synthetic Construct
EVQLVESGGGVVQPGGSLRLSCAASGFTFSSNAMSWVRQAPGKGLEWVAGISAGGSDTYYPASVKGRFTISRDNSKNTLYLQMNSLRAEDTAVYYCARETWNHLFDYWGQGTLVTVSSASTKGPSVFPLAPSSKSTSGGTAALGCLVKDYFPEPVTVSWNSGALTSGVHTFPAVLQSSGLYSLSSVVTVPSSSLGTQTYICNVNHKPSNTKVDKKVEPKSCDKTHTCPPCPAPELLGGPSVFLFPPKPKDTLMISRTPEVTCVVVDVSHEDPEVKFNWYVDGVEVHNAKTKPREEQYNSTYRVVSVLTVLHQDWLNGKEYKCKVSNKALPAPIEKTISKAKGQPREPQVYTLPPSREEMTKNQVSLTCLVKGFYPSDIAVEWESNGQPENNYKTTPPVLDSDGSFFLYSKLTVDKSRWQQGNVFSCSVMHEALHNHYTQKSLSLSPG

SEQ ID NO: 59 - protein, 447 aa, synthetic construct
  SOURCE 1..447
  REGION 1..447: NOTE = Synthetic Construct
EVQLVESGGGVVQPGGSLRLSCAASGFTFSSNAMSWVRQAPGKGLEWVAGISAGGSDTYYPASVKGRFTISRDNSKNTLYLQMNSLRAEDTAVYYCARETWNHLFDYWGQGTLVTVSSASTKGPSVFPLAPSSKSTSGGTAALGCLVKDYFPEPVTVSWNSGALTSGVHTFPAVLQSSGLYSLSSVVTVPSSSLGTQTYICNVNHKPSNTKVDKKVEPKSCDKTHTCPPCPAPEAAGAPSVFLFPPKPKDTLMISRTPEVTCVVVDVSHEDPEVKFNWYVDGVEVHNAKTKPREEQYASTYRVVSVLTVLHQDWLNGKEYKCKVSNKALPAPIEKTISKAKGQPREPQVYTLPPSREEMTKNQVSLTCLVKGFYPSDIAVEWESNGQPENNYKTTPPVLDSDGSFFLYSKLTVDKSRWQQGNVFSCSVMHEALHNHYTQKSLSLSPG

SEQ ID NO: 60 - protein, 443 aa, synthetic construct
  SOURCE 1..443
  REGION 1..443: NOTE = Synthetic Construct
EVQLVESGGGVVQPGGSLRLSCAASGFTFSSNAMSWVRQAPGKGLEWVAGISAGGSDTYYPASVKGRFTISRDNSKNTLYLQMNSLRAEDTAVYYCARETWNHLFDYWGQGTLVTVSSASTKGPSVFPLAPCSRSTSESTAALGCLVKDYFPEPVTVSWNSGALTSGVHTFPAVLQSSGLYSLSSVVTVPSSNFGTQTYTCNVDHKPSNTKVDKTVERKCCVECPPCPAPPVAGPSVFLFPPKPKDTLMISRTPEVTCVVVDVSHEDPEVQFNWYVDGVEVHNAKTKPREEQFNSTFRVVSVLTVVHQDWLNGKEYKCKVSNKGLPAPIEKTISKTKGQPREPQVYTLPPSREEMTKNQVSLTCLVKGFYPSDIAVEWESNGQPENNYKTTPPMLDSDGSFFLYSKLTVDKSRWQQGNVFSCSVMHEALHNHYTQKSLSLSPG

SEQ ID NO: 61 - protein, 443 aa, synthetic construct
  SOURCE 1..443
  REGION 1..443: NOTE = Synthetic Construct
EVQLVESGGGVVQPGGSLRLSCAASGFTFSSNAMSWVRQAPGKGLEWVAGISAGGSDTYYPASVKGRFTISRDNSKNTLYLQMNSLRAEDTAVYYCARETWNHLFDYWGQGTLVTVSSASTKGPSVFPLAPCSRSTSESTAALGCLVKDYFPEPVTVSWNSGALTSGVHTFPAVLQSSGLYSLSSVVTVPSSNFGTQTYTCNVDHKPSNTKVDKTVERKCCVECPPCPAPPVAGPSVFLFPPKPKDTLMISRTPEVTCVVVDVSHEDPEVQFNWYVDGVEVHNAKTKPREEQFNSTFRVVSVLTVVHQDWLNGKEYKCKVSNKGLPSSIEKTISKTKGQPREPQVYTLPPSREEMTKNQVSLTCLVKGFYPSDIAVEWESNGQPENNYKTTPPMLDSDGSFFLYSKLTVDKSRWQQGNVFSCSVMHEALHNHYTQKSLSLSPG

SEQ ID NO: 62 - protein, 444 aa, synthetic construct
  SOURCE 1..444
  REGION 1..444: NOTE = Synthetic Construct
EVQLVESGGGVVQPGGSLRLSCAASGFTFSSNAMSWVRQAPGKGLEWVAGISAGGSDTYYPASVKGRFTISRDNSKNTLYLQMNSLRAEDTAVYYCARETWNHLFDYWGQGTLVTVSSASTKGPSVFPLAPCSRSTSESTAALGCLVKDYFPEPVTVSWNSGALTSGVHTFPAVLQSSGLYSLSSVVTVPSSSLGTKTYTCNVDHKPSNTKVDKRVESKYGPPCPPCPAPEFLGGPSVFLFPPKPKDTLMISRTPEVTCVVVDVSQEDPEVQFNWYVDGVEVHNAKTKPREEQFNSTYRVVSVLTVLHQDWLNGKEYKCKVSNKGLPSSIEKTISKAKGQPREPQVYTLPPSQEEMTKNQVSLTCLVKGFYPSDIAVEWESNGQPENNYKTTPPVLDSDGSFFLYSRLTVDKSRWQEGNVFSCSVMHEALHNHYTQKSLSLSLG

SEQ ID NO: 63 - protein, 214 aa, synthetic construct
  SOURCE 1..214
  REGION 1..214: NOTE = Synthetic Construct
SYELTQPPSVSVSPGQTARITCSGGSYSSYYYAWYQQKPGQAPVTLIYSDDKRPSNIPERFSGSSSGTTVTLTISGVQAEDEADYYCGGYDQSSYTNPFGGGTKLTVLGQPKAAPSVTLFPPSSEELQANKATLVCLISDFYPGAVTVAWKADSSPVKAGVETTTPSKQSNNKYAASSYLSLTPEQWKSHRSYSCQVTHEGSTVEKTVAPTECS

SEQ ID NO: 64 - protein, 17 aa, synthetic construct
  SOURCE 1..17
  REGION 1..17: NOTE = Synthetic Construct
ADGSPVKAGVETTKPSK

SEQ ID NO: 65 - protein, 44 aa, synthetic construct
  SOURCE 1..44
  REGION 1..44: NOTE = Synthetic Construct
FSGSSSGTTVTLTISGVQAEDEADYYCGGYDQSSYTNPFGGGTK

SEQ ID NO: 66 - protein, 41 aa, synthetic construct
  SOURCE 1..41
  REGION 1..41: NOTE = Synthetic Construct
ITCSGGSYSSYYYAWYQQKPGQAPVTLIYSDDKRPSNIPER

SEQ ID NO: 67 - protein, 10 aa, synthetic construct
  SOURCE 1..10
  REGION 1..10: NOTE = Synthetic Construct
FGGGTKLTVL

SEQ ID NO: 68 - protein, 10 aa, synthetic construct
  SOURCE 1..10
  REGION 1..10: NOTE = Synthetic Construct
FGTGTKVTVL

SEQ ID NO: 69 - protein, 10 aa, synthetic construct
  SOURCE 1..10
  REGION 1..10: NOTE = Synthetic Construct
FGGGTQLTVL

SEQ ID NO: 70 - protein, 10 aa, synthetic construct
  SOURCE 1..10
  REGION 1..10: NOTE = Synthetic Construct
FGGGTRLTVL

SEQ ID NO: 71 - protein, 108 aa, synthetic construct
  SOURCE 1..108
  REGION 1..108: NOTE = Synthetic Construct
  VARIANT 101: NOTE = X = Gly or Thr
  VARIANT 104: NOTE = X = Lys, Gln, or Arg
  VARIANT 105: NOTE = X = Leu or Val
SYELTQPPSVSVSPGQTARITCSGGSYSSYYYAWYQQKPGQAPVTLIYSDDKRPSNIPERFSGSSSGTTVTLTISGVQAEDEADYYCGGYDQSSYTNPFGXGTXXTVL

SEQ ID NO: 72 - protein, 106 aa, synthetic construct
  SOURCE 1..106
  REGION 1..106: NOTE = Synthetic Construct
  VARIANT 63: NOTE = X = Asn, Asp, or Ser
  VARIANT 64: NOTE = X = Asp, Asn, or Ser
GQPKANPTVTLFPPSSEELQANKATLVCLISDFYPGAVTVAWKADGSPVKAGVETTKPSKQSXXKYAASSYLSLTPEQWKSHRSYSCQVTHEGSTVEKTVAPTECS

SEQ ID NO: 73 - protein, 118 aa, synthetic construct; identical to SEQ ID NO: 17
  SOURCE 1..118
  REGION 1..118: NOTE = Synthetic Construct

SEQ ID NO: 74 - protein, 107 aa, synthetic construct
  SOURCE 1..107
  REGION 1..107: NOTE = Synthetic Construct
ALTQPASVSANPGETVKIACSGGDYYSYYYGWYQQKAPGSALVTVIYSDDKRPSDIPSRFSGSASGSTATLTITGVRAEDEAVYYCGGYDYSTYANAFGAGTTLTVL

SEQ ID NO: 75 - protein, 117 aa, synthetic construct
  SOURCE 1..117
  REGION 1..117: NOTE = Synthetic Construct
DVQLVESGGGVVRPGESLRLSCEASGFTFSSNAMSWVRQAPGKGLEWVAGISSGSDTYYGDSVKGRLTISRDNSKNILYLQMNSLTAEDTAVYYCARETWNHLFDYWGLGTLVTVSS

SEQ ID NO: 76 - protein, 107 aa, synthetic construct; identical to SEQ ID NO: 18
  SOURCE 1..107
  REGION 1..107: NOTE = Synthetic Construct

SEQ ID NO: 77 - protein, 118 aa, synthetic construct; identical to SEQ ID NO: 17
  SOURCE 1..118
  REGION 1..118: NOTE = Synthetic Construct

SEQ ID NO: 78 - protein, 117 aa, synthetic construct; identical to SEQ ID NO: 75
  SOURCE 1..117
  REGION 1..117: NOTE = Synthetic Construct

SEQ ID NO: 79 - protein, 117 aa, synthetic construct
  SOURCE 1..117
  REGION 1..117: NOTE = Synthetic Construct
DVQLVESGGGVVRPGESLRLSCAVSGFRFSSYAMSWVRQAPGKGLEWVSGISSGGDTYYVDSVKGRFTISRDNSKNTLYLQVNSLTAEDTAIYYCARETWNHLFDYWGLGTLVTVSS

SEQ ID NO: 80 - protein, 118 aa, synthetic construct
  SOURCE 1..118
  REGION 1..118: NOTE = Synthetic Construct
DVQLVESGGGVVRPGESLRLSCAASGFTFSSYAMSWVRQAPGKGLEWLAGISAGGSDTYYIDSVKGRFTISRDNPKNSLYLQMSSLTAEDTAVYYCARETWNHLFDYWGLGTLVTVSS

SEQ ID NO: 81 - protein, 117 aa, synthetic construct
  SOURCE 1..117
  REGION 1..117: NOTE = Synthetic Construct
EVQLVESGGGVVQPGGSLRLSCAASGFTFSSNAMSWVRQAPGKGLEWVAGISSGSDTYYGDSVKGRFTISRDNSKNTLYLQMNSLTAEDTAVYYCARETWNHLFDYWGQGTLVTVSS

SEQ ID NO: 82 - protein, 117 aa, synthetic construct
  SOURCE 1..117
  REGION 1..117: NOTE = Synthetic Construct
EVQLVESGGGVVQPGGSLRLSCAASGFTFSSNAVSWVRQAPGKGLEWVAGISSGSDTYYGDSVKGRFTISRDNSKNTLYLQMNSLTAEDTAVYYCARETWNHLFDYWGQGTLVTVSS

SEQ ID NO: 83 - protein, 117 aa, synthetic construct
  SOURCE 1..117
  REGION 1..117: NOTE = Synthetic Construct
EVQLVESGGGVVQPGGSLRLSCAASGFRFSSYAMSWVRQAPGKGLEWVSGISSGGDTYYVDSVKGRFTISRDNSKNTLYLQMNSLRAEDTAVYYCARETWNHLFDYWGQGTLVTVSS

SEQ ID NO: 84 - protein, 117 aa, synthetic construct
  SOURCE 1..117
  REGION 1..117: NOTE = Synthetic Construct
EVQLVESGGGVVQPGGSLRLSCAASGFRFSSYAVSWVRQAPGKGLEWVSGISSGGDTYYVDSVKGRFTISRDNSKNTLYLQMNSLRAEDTAVYYCARETWNHLFDYWGQGTLVTVSS

SEQ ID NO: 85 - protein, 118 aa, synthetic construct
  SOURCE 1..118
  REGION 1..118: NOTE = Synthetic Construct
EVQLVESGGGVVQPGGSLRLSCAASGFTFSSNAVSWVRQAPGKGLEWVAGISAGGSDTYYPASVKGRFTISRDNSKNTLYLQMNSLRAEDTAVYYCARETWNHLFDYWGQGTLVTVSS

SEQ ID NO: 86 - protein, 118 aa, synthetic construct
  SOURCE 1..118
  REGION 1..118: NOTE = Synthetic Construct
EVQLVESGGGVVQPGGSLRLSCAASGFTFSSNALSWVRQAPGKGLEWVAGISAGGSDTYYPASVKGRFTISRDNSKNTLYLQMNSLRAEDTAVYYCARETWNHLFDYWGQGTLVTVSS

SEQ ID NO: 87 - protein, 117 aa, synthetic construct
  SOURCE 1..117
  REGION 1..117: NOTE = Synthetic Construct
EVQLVESGGGVVQPGGSLRLSCAASGFTFSSNALSWVRQAPGKGLEWVAGISSGSDTYYGDSVKGRFTISRDNSKNTLYLQMNSLTAEDTAVYYCARETWNHLFDYWGQGTLVTVSS

SEQ ID NO: 88 - protein, 117 aa, synthetic construct
  SOURCE 1..117
  REGION 1..117: NOTE = Synthetic Construct
EVQLVESGGGVVQPGGSLRLSCAASGFRFSSYALSWVRQAPGKGLEWVSGISSGGDTYYVDSVKGRFTISRDNSKNTLYLQMNSLRAEDTAVYYCARETWNHLFDYWGQGTLVTVSS

SEQ ID NO: 89 - protein, 117 aa, synthetic construct; identical to SEQ ID NO: 79
  SOURCE 1..117
  REGION 1..117: NOTE = Synthetic Construct

SEQ ID NO: 90 - protein, 118 aa, synthetic construct
  SOURCE 1..118
  REGION 1..118: NOTE = Synthetic Construct
DVQLVESGGAVVRPGESLRLSCAASGFTFSSYAMSWVRQAPGKGLEWLAGISAGGSDTYYIDSVKGRFTISRDNSENSLYLQMNSLTAEDTAVYYCARETWNHLFDYWGLGTLVTVSS

SEQ ID NO: 91 - protein, 119 aa, synthetic construct
  SOURCE 1..119
  REGION 1..119: NOTE = Synthetic Construct
DVQLVESGGGVVRPGESLRLSCAASGFTFSSYAMSWVRQAPGKGLEWLAGISAGGSDTYYIDSVKGRFTISRRQFQEQSLSPNEPALTAEDTAVYYCARETWNHLFDYWGLGTLVTVSS

SEQ ID NO: 92 - protein, 118 aa, synthetic construct
  SOURCE 1..118
  REGION 1..118: NOTE = Synthetic Construct
DVQLVESGGGVVRPGESLRLSCAASGFTFSSHAMSWVRQAPGKGLEWLAGISAGGSDTYYIDSVKGRFTISRDNSKSSLYLRMNSLTAEDTAVYYCARETWNHLFDYWGLGTLVTVSS

SEQ ID NO: 93 - protein, 118 aa, synthetic construct
  SOURCE 1..118
  REGION 1..118: NOTE = Synthetic Construct
DVQLVESGGGVVRPGESLRLSCAASGFTFSSNAMSWVRQAPGKGLEWLAGISAGGSDTYYPASVKGRFTISRDNPKNTLYLQMNTLTAEDTAVYYCARETWNHLFDYWGLGTLVTVSS

SEQ ID NO: 94 - protein, 118 aa, synthetic construct
  SOURCE 1..118
  REGION 1..118: NOTE = Synthetic Construct
DVQLVESGGGVVRPGESLRLSCAASGFTFSTYAMSWVRQAPGKGLEWVSGISASGSGTYYGDSVKGRFTMSRDNSKNTLYLQMNSLTAEDTAVYYCARETWNHLFDYWGLGTLVTVSS

SEQ ID NO: 95 - protein, 117 aa, synthetic construct
  SOURCE 1..117
  REGION 1..117: NOTE = Synthetic Construct
DVQLVESGGGVVRPGESLRLSCAASGFSFSSNAMSWVRQAPGKGLEWVAGISASGDTYYSGSMKGRFTISRDNSKNTLYLQMNSLTAEDTAVYYCARETWNHLFDYWGLGTLVTVSS

SEQ ID NO: 96 - protein, 117 aa, synthetic construct
  SOURCE 1..117
  REGION 1..117: NOTE = Synthetic Construct
DVQLVESGGGVVRPGESLRLSCAVSGFRFSSYAMSWVRQAPGKGLEWVSGISSDSDAYYVDSVKGRFTISRDNSKNTLYLQVNSLTAEDTAVYYCARETWNHLFDYWGLGTMVTVSS

SEQ ID NO: 97 - protein, 117 aa, synthetic construct
  SOURCE 1..117
  REGION 1..117: NOTE = Synthetic Construct
DVQLVESGGGVVRPGESLRLSCEASGFTFSSDAMSWVRQAPGKGLEWVSGISSGSSTYYGGSVKGRFTISRDNSKNTLYLQMNSLTAEDTAVYYCARETWNHLFDYWGLGTLVTVSS

SEQ ID NO: 98 - protein, 117 aa, synthetic construct; identical to SEQ ID NO: 79
  SOURCE 1..117
  REGION 1..117: NOTE = Synthetic Construct

SEQ ID NO: 99 - protein, 118 aa, synthetic construct
  SOURCE 1..118
  REGION 1..118: NOTE = Synthetic Construct
DVQLVESGGGVVRPGESLRLSCAASGFTFSSYAMSWVRQAPGKGLEWLAGISAGGSDTYYIDSVKGRFTISRDNSKNSLYLQVNSLTAEDTAVYYCARETWNHLFDYWGLGTLVTVSS

SEQ ID NO: 100 - protein, 117 aa, synthetic construct
  SOURCE 1..117
  REGION 1..117: NOTE = Synthetic Construct
DVQLVESGGGVVRPGESLRLSCAVSGFRFSSHAMSWVRQAPGKGLEWVSGISSGGDTYYVDSVKGRFTISRDNSKNTLYLQVNSLTAEDTAIYYCARETWNHLFDYWGLGTLVTVSS

SEQ ID NO: 101 - protein, 118 aa, synthetic construct
  SOURCE 1..118
  REGION 1..118: NOTE = Synthetic Construct
DVQLVDSGGGVVRPGESLRLSCAASGFTFSSYAMSWVRQAPGKGLEWLAGISAGGSDTYYIDSVKGRFTISRDNSKNSLYLQMNSLTAEDTAVYYCARETWNHLFDYWGLGTLVTVSS

SEQ ID NO: 102 - protein, 118 aa, synthetic construct
  SOURCE 1..118
  REGION 1..118: NOTE = Synthetic Construct
DVQLVESGGGVVRPGESLRLSCAASGFTFSSYAMSWVRQAPGKGLEWLAGISAGGSDTYYIDSVKGRFTISRDNSKNSLYLQMNSLTAEDTAVYYCARETWNHLFDYWGLGTLVTVSS

SEQ ID NO: 103 - protein, 118 aa, synthetic construct
  SOURCE 1..118
  REGION 1..118: NOTE = Synthetic Construct
DLQLVESGGGVVRPGESLRLSCAASGFTFSSYAMSWVRQAPGKGLEWLAGISAGGSDTYYIDSVKGRFTISRDNSKNSLYLQMNSLTAEDTAVYYCARETWNHLFDYWGLGTLVTVSS

SEQ ID NO: 104 - protein, 118 aa, synthetic construct
  SOURCE 1..118
  REGION 1..118: NOTE = Synthetic Construct
DVQLVESGGGVVRPGESLRLSCAASGFTFSSYAMSWVRQAPGKGLEWLAGISAGGSDAYYIDSVKGRFTISRDNSKNSLYLQMNSLTAEDTAVYYCARETWNHLFDYWGLGTLVTVSS

SEQ ID NO: 105 - protein, 118 aa, synthetic construct; identical to SEQ ID NO: 102
  SOURCE 1..118
  REGION 1..118: NOTE = Synthetic Construct

SEQ ID NO: 106 - protein, 117 aa, synthetic construct
  SOURCE 1..117
  REGION 1..117: NOTE = Synthetic Construct
DVQLVESGGGVVRPGESLRLSCEASGFTFSSNAMSWARQAPGKGLEWVAGISSGSDTYYGDSVKGRLTISRDNSKNILYLQMNSLTAEDTAVYYCARETWNHLFDYWGLGTLVTVSS

SEQ ID NO: 107 - protein, 118 aa, synthetic construct
  SOURCE 1..118
  REGION 1..118: NOTE = Synthetic Construct
DVQLVESGGGVVRPGESLRLSCAASGFTFSSNAMSWVRQAPGKGLEWLAGISAGDSDTYYPASVKGRFTISRDNPKNTLYLQMNTLTAEDTAVYYCARETWNHLFDYWGLGTLVTVSS

SEQ ID NO: 108 - protein, 118 aa, synthetic construct; identical to SEQ ID NO: 102
  SOURCE 1..118
  REGION 1..118: NOTE = Synthetic Construct

SEQ ID NO: 109 - protein, 118 aa, synthetic construct
  SOURCE 1..118
  REGION 1..118: NOTE = Synthetic Construct
DVQLVESGGAVVRPGETLRLSCTASGFTFSSYAMSWVRQAPGKGLEWVSGISASGSDTYYADSVKGRSTISRDNSKNTLYLRMSSLTAEDTAVYYCARETWNHLFDYWGLGTLVTVSS

SEQ ID NO: 110 - protein, 118 aa, synthetic construct; identical to SEQ ID NO: 102
  SOURCE 1..118
  REGION 1..118: NOTE = Synthetic Construct

SEQ ID NO: 111 - protein, 118 aa, synthetic construct
  SOURCE 1..118
  REGION 1..118: NOTE = Synthetic Construct
DVQLVESGGAVVRPGETLRLSCTASGFTFSSYAMSWVRQAPGKGLEWVSGISASGSDTYYADSVKGRSTISRDNSKNTLYLRMSSLTAEDTAVYYCARETWNHLFDYWGLGTLVTLSS

SEQ ID NO: 112-113 - skipped (2 entries)

SEQ ID NO: 114 - protein, 446 aa, synthetic construct
  SOURCE 1..446
  REGION 1..446: NOTE = Synthetic Construct
EVQLVESGGGVVQPGGSLRLSCAASGFTFSSNAMSWVRQAPGKGLEWVAGISSGSDTYYGDSVKGRFTISRDNSKNTLYLQMNSLTAEDTAVYYCARETWNHLFDYWGQGTLVTVSSASTKGPSVFPLAPSSKSTSGGTAALGCLVKDYFPEPVTVSWNSGALTSGVHTFPAVLQSSGLYSLSSVVTVPSSSLGTQTYICNVNHKPSNTKVDKKVEPKSCDKTHTCPPCPAPELLGGPSVFLFPPKPKDTLMISRTPEVTCVVVDVSHEDPEVKFNWYVDGVEVHNAKTKPREEQYNSTYRVVSVLTVLHQDWLNGKEYKCKVSNKALPAPIEKTISKAKGQPREPQVYTLPPSREEMTKNQVSLTCLVKGFYPSDIAVEWESNGQPENNYKTTPPVLDSDGSFFLYSKLTVDKSRWQQGNVFSCSVMHEALHNHYTQKSLSLSPG

SEQ ID NO: 115 - protein, 446 aa, synthetic construct
  SOURCE 1..446
  REGION 1..446: NOTE = Synthetic Construct
EVQLVESGGGVVQPGGSLRLSCAASGFTFSSNAMSWVRQAPGKGLEWVAGISSGSDTYYGDSVKGRFTISRDNSKNTLYLQMNSLTAEDTAVYYCARETWNHLFDYWGQGTLVTVSSASTKGPSVFPLAPSSKSTSGGTAALGCLVKDYFPEPVTVSWNSGALTSGVHTFPAVLQSSGLYSLSSVVTVPSSSLGTQTYICNVNHKPSNTKVDKKVEPKSCDKTHTCPPCPAPEAAGAPSVFLFPPKPKDTLMISRTPEVTCVVVDVSHEDPEVKFNWYVDGVEVHNAKTKPREEQYASTYRVVSVLTVLHQDWLNGKEYKCKVSNKALPAPIEKTISKAKGQPREPQVYTLPPSREEMTKNQVSLTCLVKGFYPSDIAVEWESNGQPENNYKTTPPVLDSDGSFFLYSKLTVDKSRWQQGNVFSCSVMHEALHNHYTQKSLSLSPG

SEQ ID NO: 116 - protein, 442 aa, synthetic construct
  SOURCE 1..442
  REGION 1..442: NOTE = Synthetic Construct
EVQLVESGGGVVQPGGSLRLSCAASGFTFSSNAMSWVRQAPGKGLEWVAGISSGSDTYYGDSVKGRFTISRDNSKNTLYLQMNSLTAEDTAVYYCARETWNHLFDYWGQGTLVTVSSASTKGPSVFPLAPCSRSTSESTAALGCLVKDYFPEPVTVSWNSGALTSGVHTFPAVLQSSGLYSLSSVVTVPSSNFGTQTYTCNVDHKPSNTKVDKTVERKCCVECPPCPAPPVAGPSVFLFPPKPKDTLMISRTPEVTCVVVDVSHEDPEVQFNWYVDGVEVHNAKTKPREEQFNSTFRVVSVLTVVHQDWLNGKEYKCKVSNKGLPAPIEKTISKTKGQPREPQVYTLPPSREEMTKNQVSLTCLVKGFYPSDIAVEWESNGQPENNYKTTPPMLDSDGSFFLYSKLTVDKSRWQQGNVFSCSVMHEALHNHYTQKSLSLSPG

SEQ ID NO: 117 - protein, 442 aa, synthetic construct
  SOURCE 1..442
  REGION 1..442: NOTE = Synthetic Construct
EVQLVESGGGVVQPGGSLRLSCAASGFTFSSNAMSWVRQAPGKGLEWVAGISSGSDTYYGDSVKGRFTISRDNSKNTLYLQMNSLTAEDTAVYYCARETWNHLFDYWGQGTLVTVSSASTKGPSVFPLAPCSRSTSESTAALGCLVKDYFPEPVTVSWNSGALTSGVHTFPAVLQSSGLYSLSSVVTVPSSNFGTQTYTCNVDHKPSNTKVDKTVERKCCVECPPCPAPPVAGPSVFLFPPKPKDTLMISRTPEVTCVVVDVSHEDPEVQFNWYVDGVEVHNAKTKPREEQFNSTFRVVSVLTVVHQDWLNGKEYKCKVSNKGLPSSIEKTISKTKGQPREPQVYTLPPSREEMTKNQVSLTCLVKGFYPSDIAVEWESNGQPENNYKTTPPMLDSDGSFFLYSKLTVDKSRWQQGNVFSCSVMHEALHNHYTQKSLSLSPG

SEQ ID NO: 118 - protein, 443 aa, synthetic construct
  SOURCE 1..443
  REGION 1..443: NOTE = Synthetic Construct
EVQLVESGGGVVQPGGSLRLSCAASGFTFSSNAMSWVRQAPGKGLEWVAGISSGSDTYYGDSVKGRFTISRDNSKNTLYLQMNSLTAEDTAVYYCARETWNHLFDYWGQGTLVTVSSASTKGPSVFPLAPCSRSTSESTAALGCLVKDYFPEPVTVSWNSGALTSGVHTFPAVLQSSGLYSLSSVVTVPSSSLGTKTYTCNVDHKPSNTKVDKRVESKYGPPCPPCPAPEFLGGPSVFLFPPKPKDTLMISRTPEVTCVVVDVSQEDPEVQFNWYVDGVEVHNAKTKPREEQFNSTYRVVSVLTVLHQDWLNGKEYKCKVSNKGLPSSIEKTISKAKGQPREPQVYTLPPSQEEMTKNQVSLTCLVKGFYPSDIAVEWESNGQPENNYKTTPPVLDSDGSFFLYSRLTVDKSRWQEGNVFSCSVMHEALHNHYTQKSLSLSLG

SEQ ID NO: 119 - protein, 446 aa, synthetic construct
  SOURCE 1..446
  REGION 1..446: NOTE = Synthetic Construct
EVQLVESGGGVVQPGGSLRLSCAASGFRFSSYAMSWVRQAPGKGLEWVSGISSGGDTYYVDSVKGRFTISRDNSKNTLYLQMNSLRAEDTAVYYCARETWNHLFDYWGQGTLVTVSSASTKGPSVFPLAPSSKSTSGGTAALGCLVKDYFPEPVTVSWNSGALTSGVHTFPAVLQSSGLYSLSSVVTVPSSSLGTQTYICNVNHKPSNTKVDKKVEPKSCDKTHTCPPCPAPELLGGPSVFLFPPKPKDTLMISRTPEVTCVVVDVSHEDPEVKFNWYVDGVEVHNAKTKPREEQYNSTYRVVSVLTVLHQDWLNGKEYKCKVSNKALPAPIEKTISKAKGQPREPQVYTLPPSREEMTKNQVSLTCLVKGFYPSDIAVEWESNGQPENNYKTTPPVLDSDGSFFLYSKLTVDKSRWQQGNVFSCSVMHEALHNHYTQKSLSLSPG

SEQ ID NO: 120 - protein, 446 aa, synthetic construct
  SOURCE 1..446
  REGION 1..446: NOTE = Synthetic Construct
EVQLVESGGGVVQPGGSLRLSCAASGFRFSSYAMSWVRQAPGKGLEWVSGISSGGDTYYVDSVKGRFTISRDNSKNTLYLQMNSLRAEDTAVYYCARETWNHLFDYWGQGTLVTVSSASTKGPSVFPLAPSSKSTSGGTAALGCLVKDYFPEPVTVSWNSGALTSGVHTFPAVLQSSGLYSLSSVVTVPSSSLGTQTYICNVNHKPSNTKVDKKVEPKSCDKTHTCPPCPAPEAAGAPSVFLFPPKPKDTLMISRTPEVTCVVVDVSHEDPEVKFNWYVDGVEVHNAKTKPREEQYASTYRVVSVLTVLHQDWLNGKEYKCKVSNKALPAPIEKTISKAKGQPREPQVYTLPPSREEMTKNQVSLTCLVKGFYPSDIAVEWESNGQPENNYKTTPPVLDSDGSFFLYSKLTVDKSRWQQGNVFSCSVMHEALHNHYTQKSLSLSPG

SEQ ID NO: 121 - protein, 442 aa, synthetic construct
  SOURCE 1..442
  REGION 1..442: NOTE = Synthetic Construct
EVQLVESGGGVVQPGGSLRLSCAASGFRFSSYAMSWVRQAPGKGLEWVSGISSGGDTYYVDSVKGRFTISRDNSKNTLYLQMNSLRAEDTAVYYCARETWNHLFDYWGQGTLVTVSSASTKGPSVFPLAPCSRSTSESTAALGCLVKDYFPEPVTVSWNSGALTSGVHTFPAVLQSSGLYSLSSVVTVPSSNFGTQTYTCNVDHKPSNTKVDKTVERKCCVECPPCPAPPVAGPSVFLFPPKPKDTLMISRTPEVTCVVVDVSHEDPEVQFNWYVDGVEVHNAKTKPREEQFNSTFRVVSVLTVVHQDWLNGKEYKCKVSNKGLPAPIEKTISKTKGQPREPQVYTLPPSREEMTKNQVSLTCLVKGFYPSDIAVEWESNGQPENNYKTTPPMLDSDGSFFLYSKLTVDKSRWQQGNVFSCSVMHEALHNHYTQKSLSLSPG

SEQ ID NO: 122 - protein, 442 aa, synthetic construct
  SOURCE 1..442
  REGION 1..442: NOTE = Synthetic Construct
EVQLVESGGGVVQPGGSLRLSCAASGFRFSSYAMSWVRQAPGKGLEWVSGISSGGDTYYVDSVKGRFTISRDNSKNTLYLQMNSLRAEDTAVYYCARETWNHLFDYWGQGTLVTVSSASTKGPSVFPLAPCSRSTSESTAALGCLVKDYFPEPVTVSWNSGALTSGVHTFPAVLQSSGLYSLSSVVTVPSSNFGTQTYTCNVDHKPSNTKVDKTVERKCCVECPPCPAPPVAGPSVFLFPPKPKDTLMISRTPEVTCVVVDVSHEDPEVQFNWYVDGVEVHNAKTKPREEQFNSTFRVVSVLTVVHQDWLNGKEYKCKVSNKGLPSSIEKTISKTKGQPREPQVYTLPPSREEMTKNQVSLTCLVKGFYPSDIAVEWESNGQPENNYKTTPPMLDSDGSFFLYSKLTVDKSRWQQGNVFSCSVMHEALHNHYTQKSLSLSPG

SEQ ID NO: 123 - protein, 443 aa, synthetic construct
  SOURCE 1..443
  REGION 1..443: NOTE = Synthetic Construct
EVQLVESGGGVVQPGGSLRLSCAASGFRFSSYAMSWVRQAPGKGLEWVSGISSGGDTYYVDSVKGRFTISRDNSKNTLYLQMNSLRAEDTAVYYCARETWNHLFDYWGQGTLVTVSSASTKGPSVFPLAPCSRSTSESTAALGCLVKDYFPEPVTVSWNSGALTSGVHTFPAVLQSSGLYSLSSVVTVPSSSLGTKTYTCNVDHKPSNTKVDKRVESKYGPPCPPCPAPEFLGGPSVFLFPPKPKDTLMISRTPEVTCVVVDVSQEDPEVQFNWYVDGVEVHNAKTKPREEQFNSTYRVVSVLTVLHQDWLNGKEYKCKVSNKGLPSSIEKTISKAKGQPREPQVYTLPPSQEEMTKNQVSLTCLVKGFYPSDIAVEWESNGQPENNYKTTPPVLDSDGSFFLYSRLTVDKSRWQEGNVFSCSVMHEALHNHYTQKSLSLSLG

SEQ ID NO: 124 - protein, 447 aa, synthetic construct
  SOURCE 1..447
  REGION 1..447: NOTE = Synthetic Construct
EVQLVESGGGVVQPGGSLRLSCAASGFTFSSNAMSWVRQAPGKGLEWVAGISAGGSDTYYPASVKGRFTISRDNSKNTLYLQMNSLRAEDTAVYYCARETWNHLFDYWGQGTLVTVSSASTKGPSVFPLAPSSKSTSGGTAALGCLVKDYFPEPVTVSWNSGALTSGVHTFPAVLQSSGLYSLSSVVTVPSSSLGTQTYICNVNHKPSNTKVDKKVEPKSCDKTHTCPPCPAPEAAGAPSVFLFPPKPKDTLMISRTPEVTCVVVDVSHEDPEVKFNWYVDGVEVHNAKTKPREEQYNSTYRVVSVLTVLHQDWLNGKEYKCKVSNKALPAPIEKTISKAKGQPREPQVYTLPPSREEMTKNQVSLTCLVKGFYPSDIAVEWESNGQPENNYKTTPPVLDSDGSFFLYSKLTVDKSRWQQGNVFSCSVMHEALHNHYTQKSLSLSPG

SEQ ID NO: 125 - protein, 443 aa, synthetic construct
  SOURCE 1..443
  REGION 1..443: NOTE = Synthetic Construct
EVQLVESGGGVVQPGGSLRLSCAASGFTFSSNAMSWVRQAPGKGLEWVAGISAGGSDTYYPASVKGRFTISRDNSKNTLYLQMNSLRAEDTAVYYCARETWNHLFDYWGQGTLVTVSSASTKGPSVFPLAPCSRSTSESTAALGCLVKDYFPEPVTVSWNSGALTSGVHTFPAVLQSSGLYSLSSVVTVPSSNFGTQTYTCNVDHKPSNTKVDKTVERKSCVECPPCPAPPVAGPSVFLFPPKPKDTLMISRTPEVTCVVVDVSHEDPEVQFNWYVDGVEVHNAKTKPREEQFNSTFRVVSVLTVVHQDWLNGKEYKCKVSNKGLPAPIEKTISKTKGQPREPQVYTLPPSREEMTKNQVSLTCLVKGFYPSDIAVEWESNGQPENNYKTTPPMLDSDGSFFLYSKLTVDKSRWQQGNVFSCSVMHEALHNHYTQKSLSLSPG

SEQ ID NO: 126 - protein, 443 aa, synthetic construct
  SOURCE 1..443
  REGION 1..443: NOTE = Synthetic Construct
EVQLVESGGGVVQPGGSLRLSCAASGFTFSSNAMSWVRQAPGKGLEWVAGISAGGSDTYYPASVKGRFTISRDNSKNTLYLQMNSLRAEDTAVYYCARETWNHLFDYWGQGTLVTVSSASTKGPSVFPLAPCSRSTSESTAALGCLVKDYFPEPVTVSWNSGALTSGVHTFPAVLQSSGLYSLSSVVTVPSSNFGTQTYTCNVDHKPSNTKVDKTVERKCSVECPPCPAPPVAGPSVFLFPPKPKDTLMISRTPEVTCVVVDVSHEDPEVQFNWYVDGVEVHNAKTKPREEQFNSTFRVVSVLTVVHQDWLNGKEYKCKVSNKGLPAPIEKTISKTKGQPREPQVYTLPPSREEMTKNQVSLTCLVKGFYPSDIAVEWESNGQPENNYKTTPPMLDSDGSFFLYSKLTVDKSRWQQGNVFSCSVMHEALHNHYTQKSLSLSPG

SEQ ID NO: 127 - protein, 443 aa, synthetic construct
  SOURCE 1..443
  REGION 1..443: NOTE = Synthetic Construct
EVQLVESGGGVVQPGGSLRLSCAASGFTFSSNAMSWVRQAPGKGLEWVAGISAGGSDTYYPASVKGRFTISRDNSKNTLYLQMNSLRAEDTAVYYCARETWNHLFDYWGQGTLVTVSSASTKGPSVFPLAPCSRSTSESTAALGCLVKDYFPEPVTVSWNSGALTSGVHTFPAVLQSSGLYSLSSVVTVPSSNFGTQTYTCNVDHKPSNTKVDKTVERKSCVECPPCPAPPVAGPSVFLFPPKPKDTLMISRTPEVTCVVVDVSHEDPEVQFNWYVDGVEVHNAKTKPREEQFNSTFRVVSVLTVVHQDWLNGKEYKCKVSNKGLPSSIEKTISKTKGQPREPQVYTLPPSREEMTKNQVSLTCLVKGFYPSDIAVEWESNGQPENNYKTTPPMLDSDGSFFLYSKLTVDKSRWQQGNVFSCSVMHEALHNHYTQKSLSLSPG

SEQ ID NO: 128 - protein, 443 aa, synthetic construct
  SOURCE 1..443
  REGION 1..443: NOTE = Synthetic Construct
EVQLVESGGGVVQPGGSLRLSCAASGFTFSSNAMSWVRQAPGKGLEWVAGISAGGSDTYYPASVKGRFTISRDNSKNTLYLQMNSLRAEDTAVYYCARETWNHLFDYWGQGTLVTVSSASTKGPSVFPLAPCSRSTSESTAALGCLVKDYFPEPVTVSWNSGALTSGVHTFPAVLQSSGLYSLSSVVTVPSSNFGTQTYTCNVDHKPSNTKVDKTVERKCSVECPPCPAPPVAGPSVFLFPPKPKDTLMISRTPEVTCVVVDVSHEDPEVQFNWYVDGVEVHNAKTKPREEQFNSTFRVVSVLTVVHQDWLNGKEYKCKVSNKGLPSSIEKTISKTKGQPREPQVYTLPPSREEMTKNQVSLTCLVKGFYPSDIAVEWESNGQPENNYKTTPPMLDSDGSFFLYSKLTVDKSRWQQGNVFSCSVMHEALHNHYTQKSLSLSPG

SEQ ID NO: 129 - protein, 443 aa, synthetic construct
  SOURCE 1..443
  REGION 1..443: NOTE = Synthetic Construct
EVQLVESGGGVVQPGGSLRLSCAASGFTFSSNAMSWVRQAPGKGLEWVAGISAGGSDTYYPASVKGRFTISRDNSKNTLYLQMNSLRAEDTAVYYCARETWNHLFDYWGQGTLVTVSSASTKGPSVFPLAPCSRSTSESTAALGCLVKDYFPEPVTVSWNSGALTSGVHTFPAVLQSSGLYSLSSVVTVPSSNFGTQTYTCNVDHKPSNTKVDKTVERKCCVECPPCPAPPVAGPSVFLFPPKPKDTLMISRTPEVTCVVVDVSHEDPEVQFNWYVDGVEVHNAKTKPREEQFASTFRVVSVLTVVHQDWLNGKEYKCKVSNKGLPAPIEKTISKTKGQPREPQVYTLPPSREEMTKNQVSLTCLVKGFYPSDIAVEWESNGQPENNYKTTPPMLDSDGSFFLYSKLTVDKSRWQQGNVFSCSVMHEALHNHYTQKSLSLSPG

SEQ ID NO: 130 - protein, 443 aa, synthetic construct
  SOURCE 1..443
  REGION 1..443: NOTE = Synthetic Construct
EVQLVESGGGVVQPGGSLRLSCAASGFTFSSNAMSWVRQAPGKGLEWVAGISAGGSDTYYPASVKGRFTISRDNSKNTLYLQMNSLRAEDTAVYYCARETWNHLFDYWGQGTLVTVSSASTKGPSVFPLAPCSRSTSESTAALGCLVKDYFPEPVTVSWNSGALTSGVHTFPAVLQSSGLYSLSSVVTVPSSNFGTQTYTCNVDHKPSNTKVDKTVERKSCVECPPCPAPPVAGPSVFLFPPKPKDTLMISRTPEVTCVVVDVSHEDPEVQFNWYVDGVEVHNAKTKPREEQFASTFRVVSVLTVVHQDWLNGKEYKCKVSNKGLPAPIEKTISKTKGQPREPQVYTLPPSREEMTKNQVSLTCLVKGFYPSDIAVEWESNGQPENNYKTTPPMLDSDGSFFLYSKLTVDKSRWQQGNVFSCSVMHEALHNHYTQKSLSLSPG

SEQ ID NO: 131 - protein, 443 aa, synthetic construct
  SOURCE 1..443
  REGION 1..443: NOTE = Synthetic Construct
EVQLVESGGGVVQPGGSLRLSCAASGFTFSSNAMSWVRQAPGKGLEWVAGISAGGSDTYYPASVKGRFTISRDNSKNTLYLQMNSLRAEDTAVYYCARETWNHLFDYWGQGTLVTVSSASTKGPSVFPLAPCSRSTSESTAALGCLVKDYFPEPVTVSWNSGALTSGVHTFPAVLQSSGLYSLSSVVTVPSSNFGTQTYTCNVDHKPSNTKVDKTVERKCSVECPPCPAPPVAGPSVFLFPPKPKDTLMISRTPEVTCVVVDVSHEDPEVQFNWYVDGVEVHNAKTKPREEQFASTFRVVSVLTVVHQDWLNGKEYKCKVSNKGLPAPIEKTISKTKGQPREPQVYTLPPSREEMTKNQVSLTCLVKGFYPSDIAVEWESNGQPENNYKTTPPMLDSDGSFFLYSKLTVDKSRWQQGNVFSCSVMHEALHNHYTQKSLSLSPG

SEQ ID NO: 132 - protein, 329 aa, synthetic construct
  SOURCE 1..329
  REGION 1..329: NOTE = Synthetic Construct
ASTKGPSVFPLAPSSKSTSGGTAALGCLVKDYFPEPVTVSWNSGALTSGVHTFPAVLQSSGLYSLSSVVTVPSSSLGTQTYICNVNHKPSNTKVDKKVEPKSCDKTHTCPPCPAPEAAGAPSVFLFPPKPKDTLMISRTPEVTCVVVDVSHEDPEVKFNWYVDGVEVHNAKTKPREEQYNSTYRVVSVLTVLHQDWLNGKEYKCKVSNKALPAPIEKTISKAKGQPREPQVYTLPPSREEMTKNQVSLTCLVKGFYPSDIAVEWESNGQPENNYKTTPPVLDSDGSFFLYSKLTVDKSRWQQGNVFSCSVMHEALHNHYTQKSLSLSPG

SEQ ID NO: 133 - protein, 325 aa, synthetic construct
  SOURCE 1..325
  REGION 1..325: NOTE = Synthetic Construct
ASTKGPSVFPLAPCSRSTSESTAALGCLVKDYFPEPVTVSWNSGALTSGVHTFPAVLQSSGLYSLSSVVTVPSSNFGTQTYTCNVDHKPSNTKVDKTVERKSCVECPPCPAPPVAGPSVFLFPPKPKDTLMISRTPEVTCVVVDVSHEDPEVQFNWYVDGVEVHNAKTKPREEQFNSTFRVVSVLTVVHQDWLNGKEYKCKVSNKGLPAPIEKTISKTKGQPREPQVYTLPPSREEMTKNQVSLTCLVKGFYPSDIAVEWESNGQPENNYKTTPPMLDSDGSFFLYSKLTVDKSRWQQGNVFSCSVMHEALHNHYTQKSLSLSPG

SEQ ID NO: 134 - protein, 325 aa, synthetic construct
  SOURCE 1..325
  REGION 1..325: NOTE = Synthetic Construct
ASTKGPSVFPLAPCSRSTSESTAALGCLVKDYFPEPVTVSWNSGALTSGVHTFPAVLQSSGLYSLSSVVTVPSSNFGTQTYTCNVDHKPSNTKVDKTVERKCSVECPPCPAPPVAGPSVFLFPPKPKDTLMISRTPEVTCVVVDVSHEDPEVQFNWYVDGVEVHNAKTKPREEQFNSTFRVVSVLTVVHQDWLNGKEYKCKVSNKGLPAPIEKTISKTKGQPREPQVYTLPPSREEMTKNQVSLTCLVKGFYPSDIAVEWESNGQPENNYKTTPPMLDSDGSFFLYSKLTVDKSRWQQGNVFSCSVMHEALHNHYTQKSLSLSPG

SEQ ID NO: 135 - protein, 325 aa, synthetic construct
  SOURCE 1..325
  REGION 1..325: NOTE = Synthetic Construct
ASTKGPSVFPLAPCSRSTSESTAALGCLVKDYFPEPVTVSWNSGALTSGVHTFPAVLQSSGLYSLSSVVTVPSSNFGTQTYTCNVDHKPSNTKVDKTVERKSCVECPPCPAPPVAGPSVFLFPPKPKDTLMISRTPEVTCVVVDVSHEDPEVQFNWYVDGVEVHNAKTKPREEQFNSTFRVVSVLTVVHQDWLNGKEYKCKVSNKGLPSSIEKTISKTKGQPREPQVYTLPPSREEMTKNQVSLTCLVKGFYPSDIAVEWESNGQPENNYKTTPPMLDSDGSFFLYSKLTVDKSRWQQGNVFSCSVMHEALHNHYTQKSLSLSPG

SEQ ID NO: 136 - protein, 325 aa, synthetic construct
  SOURCE 1..325
  REGION 1..325: NOTE = Synthetic Construct
ASTKGPSVFPLAPCSRSTSESTAALGCLVKDYFPEPVTVSWNSGALTSGVHTFPAVLQSSGLYSLSSVVTVPSSNFGTQTYTCNVDHKPSNTKVDKTVERKCSVECPPCPAPPVAGPSVFLFPPKPKDTLMISRTPEVTCVVVDVSHEDPEVQFNWYVDGVEVHNAKTKPREEQFNSTFRVVSVLTVVHQDWLNGKEYKCKVSNKGLPSSIEKTISKTKGQPREPQVYTLPPSREEMTKNQVSLTCLVKGFYPSDIAVEWESNGQPENNYKTTPPMLDSDGSFFLYSKLTVDKSRWQQGNVFSCSVMHEALHNHYTQKSLSLSPG

SEQ ID NO: 137 - protein, 325 aa, synthetic construct
  SOURCE 1..325
  REGION 1..325: NOTE = Synthetic Construct
ASTKGPSVFPLAPCSRSTSESTAALGCLVKDYFPEPVTVSWNSGALTSGVHTFPAVLQSSGLYSLSSVVTVPSSNFGTQTYTCNVDHKPSNTKVDKTVERKCCVECPPCPAPPVAGPSVFLFPPKPKDTLMISRTPEVTCVVVDVSHEDPEVQFNWYVDGVEVHNAKTKPREEQFASTFRVVSVLTVVHQDWLNGKEYKCKVSNKGLPAPIEKTISKTKGQPREPQVYTLPPSREEMTKNQVSLTCLVKGFYPSDIAVEWESNGQPENNYKTTPPMLDSDGSFFLYSKLTVDKSRWQQGNVFSCSVMHEALHNHYTQKSLSLSPG

SEQ ID NO: 138 - protein, 325 aa, synthetic construct
  SOURCE 1..325
  REGION 1..325: NOTE = Synthetic Construct
ASTKGPSVFPLAPCSRSTSESTAALGCLVKDYFPEPVTVSWNSGALTSGVHTFPAVLQSSGLYSLSSVVTVPSSNFGTQTYTCNVDHKPSNTKVDKTVERKSCVECPPCPAPPVAGPSVFLFPPKPKDTLMISRTPEVTCVVVDVSHEDPEVQFNWYVDGVEVHNAKTKPREEQFASTFRVVSVLTVVHQDWLNGKEYKCKVSNKGLPAPIEKTISKTKGQPREPQVYTLPPSREEMTKNQVSLTCLVKGFYPSDIAVEWESNGQPENNYKTTPPMLDSDGSFFLYSKLTVDKSRWQQGNVFSCSVMHEALHNHYTQKSLSLSPG

SEQ ID NO: 139 - protein, 325 aa, synthetic construct
  SOURCE 1..325
  REGION 1..325: NOTE = Synthetic Construct
ASTKGPSVFPLAPCSRSTSESTAALGCLVKDYFPEPVTVSWNSGALTSGVHTFPAVLQSSGLYSLSSVVTVPSSNFGTQTYTCNVDHKPSNTKVDKTVERKCSVECPPCPAPPVAGPSVFLFPPKPKDTLMISRTPEVTCVVVDVSHEDPEVQFNWYVDGVEVHNAKTKPREEQFASTFRVVSVLTVVHQDWLNGKEYKCKVSNKGLPAPIEKTISKTKGQPREPQVYTLPPSREEMTKNQVSLTCLVKGFYPSDIAVEWESNGQPENNYKTTPPMLDSDGSFFLYSKLTVDKSRWQQGNVFSCSVMHEALHNHYTQKSLSLSPG

SEQ ID NO: 140 - protein, 214 aa, synthetic construct
  REGION 1..214: NOTE = Synthetic Construct
  SOURCE 1..214
ALTQPASVSANPGETVEITCSGGSYSSYYYAWYQQKSPGSAPVTLIYSDDKRPSNIPSRFSGSASGSTATLTITGVRAEDEAVYFCGGYDQSSYTNPFGAGTTLTVLRTVAAPSVFIFPPSDEQLKSGTASVVCLLNNFYPREAKVQWKVDNALQSGNSQESVTEQDSKDSTYSLSSTLTLSKADYEKHKVYACEVTHQGLSSPVTKSFNRGEC